European Patent Specification EP 3 906 567 B1, published January 29, 2025. Title: METHOD AND APPARATUS FOR INVESTIGATING INTRA- AND/OR INTERMOLECULAR INTERACTIONS INVOLVING RNA. Applicant: CENTRE NATIONAL DE LA RECHERCHE SCIENTIFIQUE ECOLE SUPERIEURE DE PHYSIQUE ET DE CHIMIE INDUSTRIELLES DE LA VILLE DE PARIS. Application EP19305004.4. The sequence listing filed with the application follows.

SEQUENCE LISTING (4 sequences)

SEQ ID NO: 1 - DNA, 55 bp, Artificial Sequence
  F_MB Forward primer
taatacgactcactatagggagacaattgcttaagggttaagcgactaagcgtac

SEQ ID NO: 2 - DNA, 49 bp, Artificial Sequence
  R_MB reverse primer
ccactgaattgagcagacccggccggagaggatcgatcagactaatcat

SEQ ID NO: 3 - DNA, 36 bp, Artificial Sequence
  sur_DNAbiot_MB
cctctcctagctagtctgattagtagcgcancaggn

SEQ ID NO: 4 - DNA, 40 bp, Artificial Sequence
  sur_compDNA2biot_MB
ggccggagaggatcgatcagactaatcatcgcgnagnccn